European Patent Application EP 4 431 617 A1, published September 18, 2024. Title: Long-read sequencing of human immunoglobulin gene introns to define a biomarker for in vivo DNA break repair. Applicant: Max-Delbrück-Centrum für Molekulare Medizin in der Helmholtz-Gemeinschaft. The sequence listing filed with the application follows.

SEQUENCE LISTING (11 sequences)

SEQ ID NO: 1 - DNA, 27 bp, synthetic construct
  source 1..27: mol_type = other DNA; note = primer
cacccttgaaagtagcccatgccttcc

SEQ ID NO: 2 - DNA, 23 bp, synthetic construct
  source 1..23: mol_type = other DNA; note = primer
ctcagtccaacacccaccactcc

SEQ ID NO: 3 - DNA, 29 bp, synthetic construct
  source 1..29: mol_type = other DNA; note = primer
ctgcctcccagtgtcctgcattacttctg

SEQ ID NO: 4 - DNA, 24 bp, synthetic construct
  source 1..24: mol_type = other DNA; note = primer
ggagggaatgtttttgcagcagcg

SEQ ID NO: 5 - DNA, 26 bp, synthetic construct
  source 1..26: mol_type = other DNA; note = primer
ggaacgcagtgtagactcagctgagg

SEQ ID NO: 6 - DNA, 23 bp, synthetic construct
  source 1..23: mol_type = other DNA; note = primer
ggagggacccaggctaagaaggc

SEQ ID NO: 7 - DNA, 27 bp, synthetic construct
  source 1..27: mol_type = other DNA; note = primer
gcaagcagtggacccaaagacgagagg

SEQ ID NO: 8 - DNA, 24 bp, synthetic construct
  source 1..24: mol_type = other DNA; note = primer
ctgatgggggtgttgttttggctg

SEQ ID NO: 9 - DNA, 27 bp, synthetic construct
  source 1..27: mol_type = other DNA; note = primer
gggctgttgttgtagctgcaagatagg

SEQ ID NO: 10 - DNA, 25 bp, synthetic construct
  source 1..25: mol_type = other DNA; note = primer
gctcagagtgtagaggtcagactgc

SEQ ID NO: 11 - DNA, 21 bp, synthetic construct
  source 1..21: mol_type = other DNA; note = primer
gggaccccattccagtctagg